European Patent Application EP 4 282 400 A1, published November 29, 2023. Title: 一种抗菌肽液体组合物及其制剂. Applicant: 江苏普莱医药生物技术有限公司. The sequence listing filed with the application follows.

SEQUENCE LISTING (4 sequences)

SEQ ID NO: 1 - protein, 10 aa, 人工序列(Artificial Sequence)
KWKSFLKTFK

SEQ ID NO: 2 - protein, 13 aa, 人工序列(Artificial Sequence)
KTVLHTALKAISS

SEQ ID NO: 3 - protein, 26 aa, 人工序列(Artificial Sequence)
KWKSFLKTFKSAAKTVLHTALKAISS

SEQ ID NO: 4 - protein, 26 aa, 人工序列(Artificial Sequence)
KWKSFLKTFKSAAKTVLHTALKAISS